European Patent Specification EP 3 755 347 B1, published June 25, 2025. Title: UNIVERSAL ANTIGEN PRESENTING CELLS AND USES THEROF. Applicant: Board of Regents, The University of Texas System REZVANI, KATY ANG, SONNY O.T. LIU, ENLI SHPALL, ELIZABETH. The sequence listing filed with the application follows.

SEQUENCE LISTING (2 sequences)

SEQ ID NO: 1 - DNA, 8202 bp, Artificial Sequence
  CS1 Construct
aatgaaagaccccacctgtaggtttggcaagctagcttaagtaacgccattttgcaaggcatggaaaaatacataactgagaatagaaaagttcagatcaaggtcaggaacagatggaacagctgaatatgggccaaacaggatatctgtggtaagcagttcctgccccggctcagggccaagaacagatggaacagctgaatatgggccaaacaggatatctgtggtaagcagttcctgccccggctcagggccaagaacagatggtccccagatgcggtccagccctcagcagtttctagagaaccatcagatgtttccagggtgccccaaggacctgaaatgaccctgtgccttatttgaactaaccaatcagttcgcttctcgcttctgttcgcgcgcttatgctccccgagctcaataaaagagcccacaacccctcactcggggcgccagtcctccgattgactgagtcgcccgggtacccgtgtatccaataaaccctcttgcagttgcatccgacttgtggtctcgctgttccttgggagggtctcctctgagtgattgactacccgtcagcgggggtctttcatttgggggctcgtccgggatcgggagacccctgcccagggaccaccgacccaccaccgggaggtaagctggccagcaacttatctgtgtctgtccgattgtctagtgtctatgcgactgattttatgcgcctgcgtcggtactagttagctaactagctctgtatctggcggacccgtgggctggaactgacgagttcggaacacccggccgcaaccctgggagacgtcccagggacttcgggggccggctttttgtggcccgacctgagtcctaaaatcccgatcgtttaggactctttggtgcaccccccttaggcaggagggatatgtggttctggtaggagacgagaacctaaaacagttcccgcctccgtctgaatttttgctttcggtttgggaccgaagccgcgccgcgcgtcttgtctgctgcagcatcgttctgtgttgtcgctctgtctgactgtgtttctgtatttgtctgaaaatatgggcccgggctagcctgttaccactccctgctaagtttgaccttaggtcactggaaagatgtcgagcggatcgctcacaaccagtcggtagatgtcagcagaagagacgttgggttaccttctgctctgcagaatggccaacctttaacgtcggatggccgcgaggcacggcacctttaaccgagacctcatcacccaggttaagatcaaggtcttttcacctggcccgcatggacacccagaccaggtggggtacatcgtgacctgggaagccttggcttttgacccccctccctgggtcaagccctttgtacaccctaagcctccgcctcctcttcctccatccgccccgtctctcccccttggcaacctcctcgttcgaccccgcctcgatcctccctttatccagccctcactccttctctaggcgcccccatatggccatatgagatcttatatggggcacccccgccccttgtaaacttccctgaccctgacatgacaagagttactaacagcccctctctccaagctcacttacaggctctctacttagtccagcacggcaagtctggagacctctggcggcagcctaccaagaacaactggaccgaccggtggtacctcacccttgcaccgagtcggcgacacagtgtgggtccgccgacaccagactaagaacctagaacctcgctggaaaggcgaccttacacagtcctgctgaccacccccaccgccctcaaagtagacggcatcgcagcttggatacacgccgcccacgtgaaggctgccgaccccgggggtggaccatcctctagactgccatgctcgaggccggcagccccacctgcctgaccctgatctacatcctgtggcagctgaccggcagcgccgccagcggccccgtgaaggagctggtgggcagcgtgggcggcgccgtgaccttccccctgaagagcaaggtgaagcaggtggacagcatcgtgtggaccttcaacaccacccccctggtgaccatccagcccgagggcggcaccatcatcgtgacccagaacagaaacagagagagagtggacttccccgacggcggctacagcctgaagctgagcaagctgaagaagaacgacagcggcatctactacgtgggcatctacagcagcagcctgcagcagcccagcacccaggagtacgtgctgcacgtgtacgagcacctgagcaagcccaaggtgaccatgggcctgcagagcaacaagaacggcacctgcgtgaccaacctgacctgctgcatggagcacggcgaggaggacgtgatctacacctggaaggccctgggccaggccgccaacgagagccacaacggcagcatcctgcccatcagctggagatggggcgagagcgacatgaccttcatctgcgtggccagaaaccccgtgagcagaaacttcagcagccccatcctggccagaaagctgtgcgagggcgccgccgacgaccccgacagcagcatggtgctgctgtgcctgctgctggtgcccctgctgctgagcctgttcgtgctgggcctgttcctgtggttcctgaagagagagagacaggaggagtacatcgaggagaagaagagagtggacatctgcagagagacccccaacatctgcccccacagcggcgagaacaccgagtacgacaccatcccccacaccaacagaaccatcctgaaggaggaccccgccaacaccgtgtacagcaccgtggagatccccaagaagatggagaacccccacagcctgctgaccatgcccgacacccccagactgttcgcctacgagaacgtgatcggcagcacctccggcagcggcgcgcctggcagcggcgagggcagcaccaagggcatggtgagcaagggcgaggagctgttcaccggggtggtgcccatcctggtcgagctggacggcgacgtaaacggccacaagttcagcgtgtccggcgagggcgagggcgatgccacctacggcaagctgaccctgaagttcatctgcaccaccggcaagctgcccgtgccctggcccaccctcgtgaccaccctgacctacggcgtgcagtgcttcagccgctaccccgaccacatgaagcagcacgacttcttcaagtccgccatgcccgaaggctacgtccaggagcgcaccatcttcttcaaggacgacggcaactacaagacccgcgccgaggtgaagttcgagggcgacaccctggtgaaccgcatcgagctgaagggcatcgacttcaaggaggacggcaacatcctggggcacaagctggagtacaactacaacagccacaacgtctatatcatggccgacaagcagaagaacggcatcaaggtgaacttcaagatccgccacaacatcgaggacggcagcgtgcagctcgccgaccactaccagcagaacacccccatcggcgacggccccgtgctgctgcccgacaaccactacctgagcacccagtccgccctgagcaaagaccccaacgagaagcgcgatcacatggtcctgctggagttcgtgaccgccgccgggatcactctcggcatggacgagctgtacaagtgacgcgtcatcatcgatccggattagtccaatttgttaaagacaggatatcagtggtccaggctctagttttgactcaacaatatcaccagctgaagcctatagagtacgagccatagataaaataaaagattttatttagtctccagaaaaaggggggaatgaaagaccccacctgtaggtttggcaagctagcttaagtaacgccattttgcaaggcatggaaaaatacataactgagaatagagaagttcagatcaaggtcaggaacagatggaacagctgaatatgggccaaacaggatatctgtggtaagcagttcctgccccggctcagggccaagaacagatggaacagctgaatatgggccaaacaggatatctgtggtaagcagttcctgccccggctcagggccaagaacagatggtccccagatgcggtccagccctcagcagtttctagagaaccatcagatgtttccagggtgccccaaggacctgaaatgaccctgtgccttatttgaactaaccaatcagttcgcttctcgcttctgttcgcgcgcttctgctccccgagctcaataaaagagcccacaacccctcactcggggcgccagtcctccgattgactgagtcgcccgggtacccgtgtatccaataaaccctcttgcagttgcatccgacttgtggtctcgctgttccttgggagggtctcctctgagtgattgactacccgtcagcgggggtctttcacacatgcagcatgtatcaaaattaatttggttttttttcttaagtatttacattaaatggccatagtacttaaagttacattggcttccttgaaataaacatggagtattcagaatgtgtcataaatatttctaattttaagatagtatctccattggctttctactttttcttttatttttttttgtcctctgtcttccatttgttgttgttgttgtttgtttgtttgtttgttggttggttggttaagctttttttttaaagatcctacactatagttcaagctagactattagctactctgtaacccagggtgagcccttgaagtcatgggtagcctgctgttttagccttcccacatctaagattacaggtatgagctatcgcatttttggtatattgattgattgattgattgatgtgtgtgtgtgtgattgtgtttgtgtgtgtgacgctgtgaaaatgtgtgtatgggtgtgtgtgaatgtgtgtatgtatgtgtgtgtgtgagtgtgtgtgtgtgtgtgtgcatgtgtgtgtgtgtgactgtgtctatgtgtatgactgtgtgtgtgtgtgtgtgtgtggctgtgtgtgtgtgtgtgtgtgtgtgttgtgaaaaaatattctatggtagtgagagccaacgctccgggcctcaggtgtcaggttggtttttgagacagagtctttcacttagcttggaattcactggccgtcgttgcttacaacgtcgtgactgggaaaaccctggcgttacccaacttaatcgccttgcagcacatccccctgcttcgccagctggcgtaatagcgaagaggcccgcaccgatcgcccttcccaacagttgcgcagcctggcaatggcgaatggcgcctgatgcggtattttctccttacgcatctgtgcggtatttcacaccgcatagctggtgcactctcagtacaatctgctctgatgccgcatagttaagccagccccgacacccgccaacagccccgctgacgcgccctgacgggcttgtctgctcccggcatccgcttacagacaagctgtgaccgtcgctccgggagctgcatgtgtcagaggttttcaccgtcatcaccgaaacgcgcgagacgaaagggcctcgcgtgatacgcctatttttataggttaatgtcatgataataatggtttcttagacgtcaggtggcacttttcggggaaatgtgcgcggaacccctatttgtttatttttctaaatacattcaaatatgtatccgctcatgagacaataaccctgataaatgcttcaataatattgaaaaaggaagagtatgagtattcaacatttccgtgtcgcccttattcccttttttgcggcattttgccttcctgtttttgctcacccagaaacgctggtgaaagtaaaagatgctgaagatcagttgggtgcacgagtgggttacatcgaactggatctcaacagcggtaagatccttgagagttttcgccccgaagaacgttttccaatgatgagcacttttaaagttctgctatgtggcgcggtattatcccgtattgacgccgggcaagagcaactcggtcgccgcatacactattctcagaatgacttggttgagtactcaccagtcacagaaaagcatcttacggatggcatgacagtaagagaattatgcagtgctgccataaccatgagtgataacactgcggccaacttacttctgacaacgatcggaggaccgaaggagctaaccgcttttttgcacaacatgggggatcatgtaactcgccttgatcgttgggaaccggagctgaatgaagccataccaaacgacgagcgtgacaccacgatgcctgtagcaatggcaacaacgttgcgcaaactattaactggcgaactacttactctagcttcccggcaacaattaatagactggatggaggcggataaagttgcaggaccacttctgcgctcggcccttccggctggctggtttattgctgataaatctggagccggtgagcgtgggtctcgcggtatcattgcagcactggggccagatggtaagccctcccgtatcgtagttatctacacgacggggagtcaggcaactatggatgaacgaaatagacagatcgctgagataggtgcctcactgattaagcattggtaactgtcagaccaagtttactcatatatactttagattgatttaaaacttcatttttaatttaaaaggatctaggtgaagatcctttttgataatctcatgaccaaaatcccttaacgtgagttttcgttccactgagcgtcagaccccgtagaaaagatcaaaggatcttcttgagatcctttttttctgcgcgtaatctgctgcttgcaaacaaaaaaaccaccgctaccagcggtggtttgtttgccggatcaagagctaccaactctttttccgaaggtaactggcttcagcagagcgcagataccaaatactgttcttctagtgtagccgtagttaggccaccacttcaagaactctgtagcaccgcctacatacctcgctctgctaatcctgttaccagtggctgctgccagtggcgataagtcgtgtcttaccgggttggactcaagacgatagttaccggataaggcgcagcggtcgggctgaacggggggttcgtgcacacagcccagcttggagcgaacgacctacaccgaactgagatacctacagcgtgagctatgagaaagcgccacgcttcccgaagggagaaaggcggacaggtatccggtaagcggcagggtcggaacaggagagcgcacgagggagcttccagggggaaacgcctggtatctttatagtcctgtcgggtttcgccacctctgacttgagcgtcgatttttgtgatgctcgtcaggggggcggagcctatggaaaaacgccagcaacgcggcctttttacggttcctggccttttgctggccttttgctcacatgttctttcctgcgttatcccctgattctgtggataaccgtattaccgcctttgagtgagctgataccgctcgccgcagccgaacgaccgagcgcagcgagtcagtgagcgaggaagcggaagagcgcccaatacgcaaaccgcctctccccgcgcgttggccgattcattaatgcagctggcacgacaggtttcccgactggaaagcgggcagtgagcgcaacgcaattaatgtgagttagctcactgccattaggcaccccaggctttacactttatgcttccggctcgtatgttgtgtggaattgtgagcggagctaacaatttcacacaggaaacagctatgaccatgattacgccaagctttgctcttaggagtttcctgcaatacatcccaaactcaaatatataaagcatttgacttgttctatgccctagggggcggggggaaggcctaagccagctttttttaacatttaaaatgttaattccattttaaatgcacagatgtttttatttcgcataagggtttcaatgtgcatgaatgctgcaatattcctgttaccaaagctagtataaataaaaatagataaacgtggaaattacttagagtttctgtcattaacgtttccttcctcagttgacaacataaatgcgcgctgctgagcaagccagtttgcatctgtcaggatcaatttcccattatgccagtcatattaattgcactagtcaattagttgatttttatttttgacatatacatgtg

SEQ ID NO: 2 - DNA, 7935 bp, Artificial Sequence
  CD48 Construct
aatgaaagaccccacctgtaggtttggcaagctagcttaagtaacgccattttgcaaggcatggaaaaatacataactgagaatagaaaagttcagatcaaggtcaggaacagatggaacagctgaatatgggccaaacaggatatctgtggtaagcagttcctgccccggctcagggccaagaacagatggaacagctgaatatgggccaaacaggatatctgtggtaagcagttcctgccccggctcagggccaagaacagatggtccccagatgcggtccagccctcagcagtttctagagaaccatcagatgtttccagggtgccccaaggacctgaaatgaccctgtgccttatttgaactaaccaatcagttcgcttctcgcttctgttcgcgcgcttatgctccccgagctcaataaaagagcccacaacccctcactcggggcgccagtcctccgattgactgagtcgcccgggtacccgtgtatccaataaaccctcttgcagttgcatccgacttgtggtctcgctgttccttgggagggtctcctctgagtgattgactacccgtcagcgggggtctttcatttgggggctcgtccgggatcgggagacccctgcccagggaccaccgacccaccaccgggaggtaagctggccagcaacttatctgtgtctgtccgattgtctagtgtctatcgactgattttatgcgcctgcgtcggtactagttagctaactagctctgtatctggcggacccgtggctggaactgacgagttcggaacacccggccgcaaccctgggagacgtcccagggacttcgggggccgctttttgtggcccgacctgagtcctaaaatcccgatcgtttaggactctttggtgcaccccccttagcaggagggatatgtggttctggtaggagacgagaacctaaaacagttcccgcctccgtctgaatttttgctttcggtttgggaccgaagccgcgccgcgcgtcttgtctgctgcagcatcgttctgtgttgtcctctgtctgactgtgtttctgtatttgtctgaaaatatgggcccgggctagcctgttaccactccctctaagtttgaccttaggtcactggaaagatgtcgagcggatcgctcacaaccagtcggtagatgtcacagaagagacgttgggttaccttctgctctgcagaatggccaacctttaacgtcggatggccgcgagcacggcacctttaaccgagacctcatcacccaggttaagatcaaggtcttttcacctggcccgcatggacacccagaccaggtggggtacatcgtgacctgggaagccttggcttttgacccccctccctgggtcaagccctttgtacaccctaagcctccgcctcctcttcctccatccgccccgtctctcccccttgcaacctcctcgttcgaccccgcctcgatcctccctttatccagccctcactccttctctaggcgcccccatatggccatatgagatcttatatggggcacccccgccccttgtaaacttccctgaccctgacatgacaagagttactaacagcccctctctccaagctcacttacaggctctctacttagtccagcacgcaagtctggagacctctggcggcagcctaccaagaacaactggaccgaccggtggtacctcacccttcaccgagtcggcgacacagtgtgggtccgccgacaccagactaagaacctagaacctcgctggaaagcgaccttacacagtcctgctgaccacccccaccgccctcaaagtagacggcatcgcagcttggatacacgccgcccacgtgaaggctgccgaccccgggggtggaccatcctctagactgccatgctcgaggtgggtgaggatagcgtgctgatcaccgagaacatgcacatgaaactgtacatggagggcaccgtgaacgaccaccacttcaagtgcacatccgagggcgaaggcaagccctacgagggcacccagaccatgaagatcaaggtggtcgagggcggccctctccccttcgccttcgacatcctggctaccagcttcatgtacggcagcaaaacctttatcaaccacacccagggcatccccgacttctttaagcagtccttccctgagggcttcacatgggagaggatcaccacatacgaagacgggggcgtgctgaccgctacccaggacaccagcctccagaacggctgcctcatctacaacgtcaagatcaacggggtgaacttcccatccaacggccctgtgatgcagaagaaaacactcggctgggaggccagcaccgagatgctgtaccccgctgacagcggcctgagaggccatgcccagatggccctgaagctcgtgggcgggggctacctgcactgctccctcaagaccacatacagatccaagaaacccgctaagaacctcaagatgcccggcttctacttcgtggaccggagactggaaagaatcaaggaggccgacaaagagacctacgtcgagcagcacgagatggctgtggccagatactgcgacctgcctagcaaactggggcacagcggcagcacctccggcagcggcgcgcctggcagcggcgagggcagcaccaagggcgagggcaggggaagtcttctaacatgcggggacgtggaggaaaatcccgggcccatgtgcagcagaggctgggacagctgcctggccctggagctgctgctgctgcccctgagcctgctggtgaccagcatccagggccacctggtgcacatgaccgtggtgagcggcagcaacgtgaccctgaacatcagcgagagcctgcccgagaactacaagcagctgacctggttctacaccttcgaccagaagatcgtggagtgggacagcagaaagagcaagtacttcgagagcaagttcaagggcagagtgagactggacccccagagcggcgccctgtacatcagcaaggtgcagaaggaggacaacagcacctacatcatgagagtgctgaagaagaccggcaacgagcaggagtggaagatcaagctgcaggtgctggaccccgtgcccaagcccgtgatcaagatcgagaagatcgaggacatggacgacaactgctacctgaagctgagctgcgtgatccccggcgagagcgtgaactacacctggtacggcgacaagagacccttccccaaggagctgcagaacagcgtgctggagaccaccctgatgccccacaactacagcagatgctacacctgccaggtgagcaacagcgtgagcagcaagaacggcaccgtgtgcctgagccccccctgcaccctggccagaagcttcggcgtggagtggatcgccagctggctggtggtgaccgtgcccaccatcctgggcctgctgctgacctgacgcgtcatcatcgatccggattagtccaatttgttaaagacaggatatcagtggtccaggctctagttttgactcaacaatatcaccagctgaagcctatagagtacgagccatagataaaataaaagattttatttagtctccagaaaaaggggggaatgaaagaccccacctgtaggtttggcaagctagcttaagtaacgccattttgcaaggcatggaaaaatacataactgagaatagagaagttcagatcaaggtcaggaacagatggaacagctgaatatgggccaaacaggatatctgtggtaagcagttcctgccccggctcagggccaagaacagatggaacagctgaatatgggccaaacaggatatctgtggtaagcagttcctgccccggctcagggccaagaacagatggtccccagatgcggtccagccctcagcagtttctagagaaccatcagatgtttccagggtgccccaaggacctgaaatgaccctgtgccttatttgaactaaccaatcagttcgcttctcgcttctgttcgcgcgcttctgctccccgagctcaataaaagagcccacaacccctcactcggggcgccagtcctccgattgactgagtcgcccgggtacccgtgtatccaataaaccctcttgcagttgcatccgacttgtggtctcgctgttccttgggagggtctcctctgagtgattgactacccgtcagcgggggtctttcacacatgcagcatgtatcaaaattaatttggttttttttcttaagtatttacattaaatggccatagtacttaaagttacattggcttccttgaaataaacatggagtattcagaatgtgtcataaatatttctaattttaagatagtatctccattggctttctactttttcttttatttttttttgtcctctgtcttccatttgttgttgttgttgttctgtttgtttgtttgttggttggttggttaatttttttttaaagatcctacactatagttcaagctagactattagctactctgtaacccagggtgaccttgaagtcatgggtagcctgctgttttagccttccccacatctaagattacaggtatgagctatcatttttggtatattgattgattgattgattgatgtgtgtgtgtgtgattgtgtttgtgtgtgtgactgtgaaaatgtgtgtatgggtgtgtgtgaatgtgtgctatgtatgtgtgtgtgtgagtgtgtgtgtgtgtgtgtgcatgtgtgtgtgtgtgactgtgtctatgctgtatgactgtgtgtgtgtgtgtgtgtgtgtgtgtgtgtgtgtgtgtgtgtgtgttgtgaaaaaatcattctatggtagtgagagccaacgctccggctcaggtgtcaggttggtttttgagacagagtctttccacttagcttggaattcactggccgtcgttttacaacgtcgtgactgggaaaaccctggcgttacccaacttaatcgccttgcagcacatccccctttcgccagctggcgtaatagcgaagaggcccgcacccgatcgcccttcccaacagttgcgcagcctgaatggcgaatggcgcctgatgcggtattttctccttcacgcatctgtgcggtatttcacaccgcatatggtgcactctcagtacaatctgctctgatgccgcatagttaagccagccccgacacccgccaacacccgctgacgcgccctgacgggcttgtctgctcccgcgcatccgcttacagacaagctgtgaccgtctccgggagctgcatgtgtcagaggttttcaccgtcatcaccgaaacgcgcgagacgaaagggcctcgtgatacgcctatttttataggttaatgtcatgatacataatggtttcttagacgtcaggtggcacttttcggggaaatgtgcgcggaacccctatttgtttatttttctaaatacattcaaatatgtatccgctcatgagacaataaccctgataaatgcttcaataatattgaaaaaggaagagtatgagtattcaacatttccgtgtcgcccttattcccttttttgcggcattttgccttcctgtttttgctcacccagaaacgctggtgaaagtaaaagatgctgaagatcagttgggtgcacgagtgggttacatcgaactggatctcaacagcggtaagatccttgagagttttcgccccgaagaacgttttccaatgatgagcacttttaaagttctgctatgtggcgcggtattatcccgtattgacgccgggcaagagcaactcggtcgccgcatacactattctcagaatgacttggttgagtactcaccagtcacagaaaagcatcttacggatggcatgacagtaagagaattatgcagtgctgccataaccatgagtgataacactgcggccaacttacttctgacaacgatcggaggaccgaaggagctaaccgcttttttgcacaacatgggggatcatgtaactcgccttgatcgttgggaaccggagctgaatgaagccataccaaacgacgagcgtgacaccacgatgcctgtagcaatggcaacaacgttgcgcaaactattaactggcgaactacttactctagcttcccggcaacaattaatagactggatggaggcggataaagttgcaggaccacttctgcgctcggcccttccggctggctggtttattgctgataaatctggagccggtgagcgtgggtctcgcggtatcattgcagcactggggccagatggtaagccctcccgtatcgtagttatctacacgacggggagtcaggcaactatggatgaacgaaatagacagatcgctgagataggtgcctcactgattaagcattggtaactgtcagaccaagtttactcatatatactttagattgatttaaaacttcatttttaatttaaaaggatctaggtgaagatcctttttgataatctcatgaccaaaatcccttaacgtgagttttcgttccactgagcgtcagaccccgtagaaaagatcaaaggatcttcttgagatcctttttttctgcgcgtaatctgctgcttgcaaacaaaaaaaccaccgctaccagcggtggtttgtttgccggatcaagagctaccaactctttttccgaaggtaactggcttcagcagagcgcagataccaaatactgttcttctagtgtagccgtagttaggccaccacttcaagaactctgtagcaccgcctacatacctcgctctgctaatcctgttaccagtggctgctgccagtggcgataagtcgtgtcttaccgggttggactcaagacgatagttaccggataaggcgcagcggtcgggctgaacggggggttcgtgcacacagcccagcttggagcgaacgacctacaccgaactgagatacctacagcgtgagctatgagaaagcgccacgcttcccgaagggagaaaggcggacaggtatccggtaagcggcagggtcggaacaggagagcgcacgagggagcttccagggggaaacgcctggtatctttatagtcctgtcgggtttcgccacctctgacttgagcgtcgatttttgtgatgctcgtcaggggggcggagcctatggaaaaacgccagcaacgcggcctttttacggttcctggccttttgctggccttttgctcacatgttctttcctgcgttatccccctgattctgtggataaccgtattaccgcctttgagtgagctgataccgctcgccgcagccgaacgcaccgagcgcagcgagtcagtgagcgaggaagcggaagagcgcccaatacgcaaaccgcctctcccccgcgcgttggccgattcattaatgcagctggcacgacaggtttcccgactggaaagcgggcagtgagcgcaacgcaattaatgtgagttagctcactcattaggcaccccaggctttacactttatgcttccgcgctcgtatgttgtgtggaattgtgagcggataacaatttcacacaggaaacagctatgaccatgatctacgccaagctttgctcttaggagtttcctaatacatcccaaactcaaatatataaagcatttgacttgttctatgccctagggggcggggggaagctaagccagctttttttaacatttaaaatgttaattcccattttaaatgcacagatgtttttatttcataagggtttcaatgtgcatgaatgctgcaatattccctgttaccaaagctagtataaataaaaatagataaacgtggaaattacttagagtttctgtcattacacgtttccttcctcagttgacaacataaatgcgctgctgagcaagccagtttgcatctgtcaggatccaatttcccattatgccagtcatattaattactagtcaattagttgatttttatttttgacatatacatgtg